European Patent Specification EP 3 976 830 B1, published May 21, 2025. Title: DETECTION OF HYPERMETHYLATED GENES FOR DIAGNOSING PANCREATIC CANCER. Applicant: Université de Paris Centre National de la Recherche Scientifique (CNRS) ASSISTANCE PUBLIQUE-HOPITAUX DE PARIS (AP-HP) INSTITUT NATIONAL DE LA SANTE ET DE LA RECHERCHE MEDICALE. The sequence listing filed with the application follows.

SEQUENCE LISTING (10 sequences)

SEQ ID NO: 1 - DNA, 1001 bp, Homo sapiens
  POU4F1 chr13: 79176072-79177072
cgccgccgatgccgctgccacctgcccggccgccgccgccgccgctgccgctgccgcgccgtggtgcgccgccgccgccaccagcccggggtgcggcagcccggacggcatgttcatggcggccgccgccgcggggtgcgacaggtggcccaggctgtgcatatgcgggtgagggtgcgcggagccgcccaggagcccgccgcccgggccgccgccgccgccccccgggccgccaccgccgcctcccccggggccgccgcccgggccgccgccgccgcccgggccgccaccgccccccgggccgtcgtgggcgccgccgccgccggccgccgcgcccgcgccgcccgcgccggccatgagcgcgagcgacggcgaggagatgtggtccagcagatcgccgggttcgagcgcctggtggtggtggtggtggtggtggtggtgcgccagaggcaccgtggaagtggacgtgcacggcacgctgttcatcgtgtggtacgtggcgtccggcttgaaaggatggctcttgccctgggacacggcgatgtccacggccgccagcgcctcggcccgcgccagcagcgtctcgtccaggctggcgaagaggttgctctgcagctgcaggcgacacaaaccaaaccaaaaaaaccacaaaaccaaaagagcaaaacaaaacaacagaagaaacacacacacaggccggaaagcacagcatgcgaagggcaaacacaaagcaaccaaaataacaacgggtttgggggcagtggagagcgggaaagacggagagggggcacattgacgaccagggagggggcagacgagaagggatgggagcgtggagagggggacagaagtagggagaaagggggacacaagaacacattccggaaacgggcgtgggagacgaaaaagagggaaaagaagaaatggaaatgtaactcgcagctggggacccgtgtcacacacccgagcacgcacagagactgcctttctgaggcgtgaaa

SEQ ID NO: 2 - DNA, 201 bp, Homo sapiens
  POU4F1 chr13: 79176472-79176672
ggttcgagcgcctggtggtggtggtggtggtggtggtggtgcgccagaggcaccgtggaagtggacgtgcacggcacgctgttcatcgtgtggtacgtggcgtccggcttgaaaggatggctcttgccctgggacacggcgatgtccacggccgccagcgcctcggcccgcgccagcagcgtctcgtccaggctggcgaag

SEQ ID NO: 3 - DNA, 1026 bp, Homo sapiens
  HOXD8 chr2: 176994063-176995088
accacttcgatatgccccaactcaaatgcacggtccggtccgtcaacacctcttgtccacgttccctgggctgcacccgcgtgtccagagctgcaaaagccacgggcaacctctgcttttgcagccaggggctcggggaggcagtcatttgctccgcagcctcctgggagtggcctccttggctcccccaagtctaaggctccgccgcggcccctccctgccggctgcgatccgcattcccgcggccccggggcacacggagcccttggcagtgcgtctttatgggccccctttaaggccggcggaggcatctcgggccgggcgcggcgctccgtccgtcggccgtagcgactgaactgcgcgcggatccctccgcggggctcctcgtccccgtcacgctgactttccgtgcagtgctgtggtgcgaaaatgcctcgccggtgcgcaccgggtcggcagcctcggcggcgggggcgagattggcgggaggggggcgcggggggggcgcggtaagaggtggcggcgggcagagggtgttttttttcttttccctccagagccggggtttgtaaaccgaggccagagtgtccccgtgggccgagcgcacttttttcttgtccgggtgcgctcagtcactggtgcctgagaggaaacagtggaggcagcggggcaggtcgcctggggcgtcggcgattatattgcggccgagccggggcgcgccgggaaaggccgggagggcggcggcgcgcgggggctgggcgaggccccgcgacccgcgagggaggcggcgcgaagccgaggcggcgggcgcaagagccgggcatgagcgcccagtagctgagcgcccgcggctgcctggcctcagaagcgacgcgcgagcgcgggcgggcggcagcagcgacgtagcccggcggtcccggcggcgagagcagccgccccacaggcccccgcggcagtgcggccgagtcgaggctcgctctctggctgcttagcgccgcccgcccgcccggggccgccgccgctgac

SEQ ID NO: 4 - DNA, 726 bp, Homo sapiens
  HOXD8 chr2: 176994363-176995088
ggcggaggcatctcgggccgggcgcggcgctccgtccgtcggccgtagcgactgaactgcgcgcggatccctccgcggggctcctcgtccccgtcacgctgactttccgtgcagtgctgtggtgcgaaaatgcctcgccggtgcgcaccgggtcggcagcctcggcggcgggggcgagattggcgggaggggggcgcggggggggcgcggtaagaggtggcggcgggcagagggtgttttttttcttttccctccagagccggggtttgtaaaccgaggccagagtgtccccgtgggccgagcgcacttttttcttgtccgggtgcgctcagtcactggtgcctgagaggaaacagtggaggcagcggggcaggtcgcctggggcgtcggcgattatattgcggccgagccggggcgcgccgggaaaggccgggagggcggcggcgcgcgggggctgggcgaggccccgcgacccgcgagggaggcggcgcgaagccgaggcggcgggcgcaagagccgggcatgagcgcccagtagctgagcgcccgcggctgcctggcctcagaagcgacgcgcgagcgcgggcgggcggcagcagcgacgtagcccggcggtcccggcggcgagagcagccgccccacaggcccccgcggcagtgcggccgagtcgaggctcgctctctggctgcttagcgccgcccgcccgcccggggccgccgccgctgac

SEQ ID NO: 5 - DNA, 20 bp, Artificial Sequence
  Forward Primer POU4F1
tggtgcgttagaggtatcgt

SEQ ID NO: 6 - DNA, 20 bp, Artificial Sequence
  Reverse Primer POU4F1
aaaccatcctttcaaaccga

SEQ ID NO: 7 - DNA, 21 bp, Artificial Sequence
  Forward Primer HOXD8
agagtcggggtttgtaaatcg

SEQ ID NO: 8 - DNA, 24 bp, Artificial Sequence
  Reverse Primer HOXD8
ctctcaaacaccaataactaaacg

SEQ ID NO: 9 - DNA, 20 bp, Artificial Sequence
  Probe POU4F1: FAM - SEQ ID NO:9 -MGB - NFQ
caacgtaccgtacacgtcca

SEQ ID NO: 10 - DNA, 16 bp, Artificial Sequence
  Probe HOXD8: FAM - SEQ ID NO:10 -MGB - NFQ
tcgtgggtcgagcgta